European Patent Application EP 4 353 816 A1, published April 17, 2024. Title: METHODS FOR PRODUCING SINOATRIAL NODE CELLS. Applicant: Academisch Medisch Centrum. Application EP. The sequence listing filed with the application follows.

SEQUENCE LISTING (22 sequences)

SEQ ID NO: 1 - DNA, 21 bp, synthetic construct
  misc_feature 1..21: note = RPLP0 FW
  source 1..21: mol_type = other DNA
atccagcaggtgttcgacaat

SEQ ID NO: 2 - DNA, 20 bp, synthetic construct
  misc_feature 1..20: note = RPLP0 RV
  source 1..20: mol_type = other DNA
gccaggactcgtttgtaccc

SEQ ID NO: 3 - DNA, 20 bp, synthetic construct
  misc_feature 1..20: note = GUSB FW
  source 1..20: mol_type = other DNA
cctgcgtcccacctagaatc

SEQ ID NO: 4 - DNA, 19 bp, synthetic construct
  misc_feature 1..19: note = GUSB RV
  source 1..19: mol_type = other DNA
atacggagcccccttgtct

SEQ ID NO: 5 - DNA, 18 bp, synthetic construct
  misc_feature 1..18: note = MESP1 FW
  source 1..18: mol_type = other DNA
gaagggcaggcgatggag

SEQ ID NO: 6 - DNA, 20 bp, synthetic construct
  misc_feature 1..20: note = MESP1 RV
  source 1..20: mol_type = other DNA
caggtctccaacagagccag

SEQ ID NO: 7 - DNA, 20 bp, synthetic construct
  misc_feature 1..20: note = TBX5 FW
  source 1..20: mol_type = other DNA
acatggagctgcacagaatg

SEQ ID NO: 8 - DNA, 20 bp, synthetic construct
  misc_feature 1..20: note = TBX5 RV
  source 1..20: mol_type = other DNA
tgctgaaaggactgtggttg

SEQ ID NO: 9 - DNA, 20 bp, synthetic construct
  misc_feature 1..20: note = TBX18 FW
  source 1..20: mol_type = other DNA
ttgctaaaggcttccgagac

SEQ ID NO: 10 - DNA, 20 bp, synthetic construct
  misc_feature 1..20: note = TBX18 RV
  source 1..20: mol_type = other DNA
aggtggaggaacttgcattg

SEQ ID NO: 11 - DNA, 24 bp, synthetic construct
  misc_feature 1..24: note = SHOX2 FW
  source 1..24: mol_type = other DNA
ccataaaggtgttctcataggggc

SEQ ID NO: 12 - DNA, 20 bp, synthetic construct
  misc_feature 1..20: note = SHOX2 RV
  source 1..20: mol_type = other DNA
aacctgaaaggacaagggcg

SEQ ID NO: 13 - DNA, 22 bp, synthetic construct
  misc_feature 1..22: note = NTM FW
  source 1..22: mol_type = other DNA
catcatgctatttggtccaggc

SEQ ID NO: 14 - DNA, 20 bp, synthetic construct
  misc_feature 1..20: note = NTM RV
  source 1..20: mol_type = other DNA
gggaagtggcactcacatca

SEQ ID NO: 15 - DNA, 22 bp, synthetic construct
  misc_feature 1..22: note = VSNL1 FW
  source 1..22: mol_type = other DNA
ggaagcagaatagcaaactggc

SEQ ID NO: 16 - DNA, 22 bp, synthetic construct
  misc_feature 1..22: note = VSNL1 RV
  source 1..22: mol_type = other DNA
gaggcgtctccataaggaaaga

SEQ ID NO: 17 - DNA, 20 bp, synthetic construct
  misc_feature 1..20: note = FLRT3 FW
  source 1..20: mol_type = other DNA
agacgggggagggctattac

SEQ ID NO: 18 - DNA, 21 bp, synthetic construct
  misc_feature 1..21: note = FLRT3 RV
  source 1..21: mol_type = other DNA
ggtcagcagtgttgaggtctt

SEQ ID NO: 19 - DNA, 21 bp, synthetic construct
  misc_feature 1..21: note = NPPA FW
  source 1..21: mol_type = other DNA
cgatctgccctcctaaaaagc

SEQ ID NO: 20 - DNA, 21 bp, synthetic construct
  misc_feature 1..21: note = NPPA RV
  source 1..21: mol_type = other DNA
ttgtcctccctggctgttatc

SEQ ID NO: 21 - DNA, 22 bp, synthetic construct
  misc_feature 1..22: note = ADM FW
  source 1..22: mol_type = other DNA
ttggcagatcactctcttagca

SEQ ID NO: 22 - DNA, 19 bp, synthetic construct
  misc_feature 1..19: note = ADM RV
  source 1..19: mol_type = other DNA
gacatccgcagttccctct